European Patent Application EP 4 813 406 A1, published September 30, 2026. Title: 一种mRNA疫苗及其应用. Applicant: 长春百克生物科技股份公司. The sequence listing filed with the application follows.

SEQUENCE LISTING (6 sequences)

SEQ ID NO: 1 - protein, 575 aa, synthetic construct
MELLILKANAITTILTAVTFCFASGQNITEEFYQSTCSAVSKGYLSALRTGWYTSVITIELSNIKENKCNGTDAKVKLIKQELDKYKNAVTELQLLMQSTPATNNRARRELPRFMNYTLNNAKKTNVTLSKKRKRRFLGFLLGVGSAIASGVAVCKVLHLEGEVNKIKSALLSTNKAVVSLSNGVSVLTFKVLDLKNYIDKQLLPILNKQSCSISNIETVIEFQQKNNRLLEITREFSVNAGVTTPVSTYMLTNSELLSLINDMPITNDQKKLMSNNVQIVRQQSYSIMCIIKEEVLAYVVQLPLYGVIDTPCWKLHTSPLCTTNTKEGSNICLTRTDRGWYCDNAGSVSFFPQAETCKVQSNRVFCDTMNSLTLPSEVNLCNVDIFNPKYDCKIMTSKTDVSSSVITSLGAIVSCYGKTKCTASNKNRGIIKTFSNGCDYVSNKGVDTVSVGNTLYYVNKQEGKSLYVKGEPIINFYDPLVFPSDEFDASISQVNEKINQSLAFIRKSDELLHNVNAGKSTTNTGFIIVIILIAVLGSSMILVSIFIIIKKTKKQTGAPPELSGVTNNGFIPHS

SEQ ID NO: 2 - protein, 254 aa, synthetic construct
MESYLVDTYQGIPYTAAVQVDLIEKDLLPASLTIWFPLFQANTPPAVLLDQLKTLTITTLYAASQNGPILKVNASAQGAAMSVLPKKFEVNATVALDEYSKLEFDKLTVCEVKTVYLTTMKPYGMVSKFVSSAKSVGKKTHDLIALCDFMDLEKNTPVTIPAFIKSVSIKESESATVEAAISSEADQALTQAKIAPYAGLIMIMTMNNPKGIFKKLGAGTQVIVELGAYVQAESISKICKTWSHQGTRYVLKSR

SEQ ID NO: 3 - DNA, 626 bp, synthetic construct
  source 1..626: mol_type = other DNA
ttaaaacagcggatgggtaccccaccatccgacccactgggtgtagtactctggtacttcgtacctttgtacgcctgttcttcccattgtacccttcctgaacttccaacccaagtaacgttagaagctcaacatttagtacaacaggaagcaccacatccagtggtgtttagtacaagcacttctgtttccccggagcgaggtataggctgtacccactgccaaaaacctttaaccgttatccgccaaccaactacgtaaaagctagtagtattatgtttttaactaggcgttcgatcaggtggatttcccctccactagtttggtcgatgaggctaggaattccccacgggtgaccgtgtcctagcctgcgtggcggccaacccagcttatgctgggacgcctttttatagacatggtgtgaagactcgcatgtgcttggttgtgattcctccggcccctgaatgcggctaaccttaaccctggagccttgtgtcacaaaccagtgatgataaggtcgtaatgagcaattccgggacgggaccgactactttgggtgtccgtgtttcttatttttcttattattgtcttatggtcacagcatatatataacatatactgtgatc

SEQ ID NO: 4 - DNA, 4773 bp, synthetic construct
  source 1..4773: mol_type = other DNA
aaataagagagaaaagaagagtaagaagaaatataagagccaccatggaactgctgatactgaaggccaacgcaatcaccaccatcctgaccgccgtgaccttctgcttcgccagcggccagaacatcaccgaggagttctaccagagcacctgcagcgccgtgagcaagggctacctgagcgccctgaggaccggctggtacaccagcgtgatcaccatcgagctgagcaacatcaaggagaacaagtgcaacggcaccgacgccaaggtgaagctgatcaagcaggagctggacaagtacaagaacgccgtgaccgagctgcagctgctgatgcagagcacccccgccaccaacaacagggccaggagggagctgcccaggttcatgaactacaccctgaacaacgccaagaagaccaacgtgaccctgagcaagaagaggaagaggaggttcctgggcttcctgctgggcgtgggcagcgccatcgccagcggcgtggccgtgtgcaaggtgctgcacctggagggcgaggtgaacaagatcaagagcgccctgctgagcaccaacaaggccgtggtgagcctgagcaacggcgtgagcgtgctgaccttcaaggtgctggacctgaagaactacatcgacaagcagctgctgcccatcctgaacaagcagagctgcagcatcagcaacatcgagacagtgatcgagttccagcagaagaacaacaggctgctggagatcaccagggagttcagcgtgaacgccggcgtgaccacccccgtgagcacctacatgctgaccaacagcgagctgctgagcctgatcaacgacatgcccatcaccaacgaccagaagaagctgatgagcaacaacgtgcagatcgtgaggcagcagagctacagcatcatgtgcatcatcaaggaggaggtgctggcctacgtggtgcagctgcccctgtacggcgtgatcgacaccccctgctggaagctgcacaccagccccctgtgcaccaccaacaccaaggagggcagcaacatctgcctgaccaggaccgacaggggctggtactgcgacaacgccggcagcgtgagcttcttcccccaggccgagacatgcaaggtgcagagcaacagggtgttctgcgacaccatgaacagcctgaccctgcccagcgaggtgaacctgtgcaacgtggacatcttcaaccccaagtacgactgcaagatcatgaccagcaagaccgacgtgagcagcagcgtgatcaccagcctgggcgccatcgtgagctgctacggcaagaccaagtgcaccgccagcaacaagaacaggggcatcatcaagaccttcagcaacggctgcgactacgtgagcaacaagggcgtggacaccgtgagcgtgggcaacaccctgtactacgtgaacaagcaggagggcaagagcctgtacgtgaagggcgagcccatcatcaacttctacgaccccctggtgttccccagcgacgagttcgacgccagcatcagccaggtgaacgagaagatcaaccagagcctggccttcatcaggaagagcgacgagctgctgcacaacgtgaacgccggcaagagcaccaccaacaccggcttcatcatcgtgatcatcctgatcgccgtgctgggcagcagcatgatcctggtgagcatcttcatcatcatcaagaagaccaagaagcagaccggcgccccccccgagctgagcggcgtgaccaacaacggcttcatcccccacagctgattaaaacagcggatgggtaccccaccatccgacccactgggtgtagtactctggtacttcgtacctttgtacgcctgttcttcccattgtacccttcctgaacttccaacccaagtaacgttagaagctcaacatttagtacaacaggaagcaccacatccagtggtgtttagtacaagcacttctgtttccccggagcgaggtataggctgtacccactgccaaaaacctttaaccgttatccgccaaccaactacgtaaaagctagtagtattatgtttttaactaggcgttcgatcaggtggatttcccctccactagtttggtcgatgaggctaggaattccccacgggtgaccgtgtcctagcctgcgtggcggccaacccagcttatgctgggacgcctttttatagacatggtgtgaagactcgcatgtgcttggttgtgattcctccggcccctgaatgcggctaaccttaaccctggagccttgtgtcacaaaccagtgatgataaggtcgtaatgagcaattccgggacgggaccgactactttgggtgtccgtgtttcttatttttcttattattgtcttatggtcacagcatatatataacatatactgtgatcatggagtcctaccttgttgatacctaccagggaattccttacacagctgctgtgcaagtggacctgattgaaaaggacctcctgcccgcctccctgaccatttggttccccctgttccaggccaacacacctcctgctgtcctgctggaccagctgaaaaccctcaccatcaccaccctgtatgcagcctctcagaatggccccatcctcaaggtgaatgccagcgcccagggggccgccatgagcgtgctccccaaaaagtttgaagtgaacgccaccgtggccttggatgaatattccaaactggagtttgacaagctcactgtgtgtgaggtgaagaccgtgtacctgaccacaatgaagccctatggcatggtgagcaaatttgtgagcagcgccaagtcagtgggcaagaaaacacatgatctcatcgccctgtgtgacttcatggacttggagaagaacacccctgtgaccattccagccttcatcaagtctgtgtccatcaaagaatctgaaagcgccacagtggaagctgccatctcctctgaggccgatcaggctctgacccaagccaaaattgccccctatgcaggcctgatcatgatcatgaccatgaacaaccccaagggcatcttcaagaagctgggggctgggacccaggtgattgtggagctgggcgcctacgtgcaggcagagagcatcagcaagatctgcaagacatggagccaccagggcacccgctacgtgctgaagagcaggtgattaaaacagcggatgggtaccccaccatccgacccactgggtgtagtactctggtacttcgtacctttgtacgcctgttcttcccattgtacccttcctgaacttccaacccaagtaacgttagaagctcaacatttagtacaacaggaagcaccacatccagtggtgtttagtacaagcacttctgtttccccggagcgaggtataggctgtacccactgccaaaaacctttaaccgttatccgccaaccaactacgtaaaagctagtagtattatgtttttaactaggcgttcgatcaggtggatttcccctccactagtttggtcgatgaggctaggaattccccacgggtgaccgtgtcctagcctgcgtggcggccaacccagcttatgctgggacgcctttttatagacatggtgtgaagactcgcatgtgcttggttgtgattcctccggcccctgaatgcggctaaccttaaccctggagccttgtgtcacaaaccagtgatgataaggtcgtaatgagcaattccgggacgggaccgactactttgggtgtccgtgtttcttatttttcttattattgtcttatggtcacagcatatatataacatatactgtgatcatggagagctacctggtggacacctaccagggcatcccctacaccgccgccgtgcaggtggacctgatcgagaaggacctgctgcccgccagcctgaccatctggttccccctgttccaggccaacaccccccccgccgtgctgctggaccagctgaagaccctgaccatcaccaccctgtacgccgccagccagaacggccccatcctgaaggtgaacgccagcgcccagggcgccgccatgagcgtgctgcccaagaagttcgaggtgaacgccaccgtggccctggacgagtacagcaagctggagttcgacaagctgaccgtgtgcgaggtgaagaccgtgtacctgaccaccatgaagccctacggcatggtgagcaagttcgtgagcagcgccaagagcgtgggcaagaagacccacgacctgatcgccctgtgcgacttcatggacctggagaagaacacccccgtgaccatccccgccttcatcaagagcgtgagcatcaaggagagcgagagcgccaccgtggaggccgccatcagcagcgaggccgaccaggccctgacccaggccaagatcgccccctacgccggcctgatcatgatcatgaccatgaacaaccccaagggcatcttcaagaagctgggcgccggcacccaggtgatcgtggagctgggcgcctacgtgcaggccgagagcatcagcaagatctgcaagacctggagccaccagggcaccaggtacgtgctgaagagcaggtaagcggccgcttaattaagctgccttctgcggggcttgccttctggccatgcccttcttctctcccttgcacctgtacctcttggtctttgaataaagcctgagtaggaagaaaaaaaaaaaaaaaaaaaaaaaaaaaaaagcatatgactaaaaaaaaaaaaaaaaaaaaaaaaaaaaaaaaaaaaaaaaaaaaaaaaaaaaaaaaaaaaaaaaaaaaaa

SEQ ID NO: 5 - DNA, 4969 bp, synthetic construct
  source 1..4969: mol_type = other DNA
gagaataaactagtattcttctggtccccacagactcagagagaacccgccaccatggaactcctcatcctgaaagccaacgccatcaccaccatcctgaccgccgtgaccttctgcttcgccagcggccagaacatcaccgaggagttctaccagagcacctgcagcgccgtgagcaagggctacctgagcgccctgaggaccggctggtacaccagcgtgatcaccatcgagctgagcaacatcaaggagaacaagtgcaacggcaccgacgccaaggtgaagctgatcaagcaggagctggacaagtacaagaacgccgtgaccgagctgcagctgctgatgcagagcacccccgccaccaacaacagggccaggagggagctgcccaggttcatgaactacaccctgaacaacgccaagaagaccaacgtgaccctgagcaagaagaggaagaggaggttcctgggcttcctgctgggcgtgggcagcgccatcgccagcggcgtggccgtgtgcaaggtgctgcacctggagggcgaggtgaacaagatcaagagcgccctgctgagcaccaacaaggccgtggtgagcctgagcaacggcgtgagcgtgctgaccttcaaggtgctggacctgaagaactacatcgacaagcagctgctgcccatcctgaacaagcagagctgcagcatcagcaacatcgagacagtgatcgagttccagcagaagaacaacaggctgctggagatcaccagggagttcagcgtgaacgccggcgtgaccacccccgtgagcacctacatgctgaccaacagcgagctgctgagcctgatcaacgacatgcccatcaccaacgaccagaagaagctgatgagcaacaacgtgcagatcgtgaggcagcagagctacagcatcatgtgcatcatcaaggaggaggtgctggcctacgtggtgcagctgcccctgtacggcgtgatcgacaccccctgctggaagctgcacaccagccccctgtgcaccaccaacaccaaggagggcagcaacatctgcctgaccaggaccgacaggggctggtactgcgacaacgccggcagcgtgagcttcttcccccaggccgagacatgcaaggtgcagagcaacagggtgttctgcgacaccatgaacagcctgaccctgcccagcgaggtgaacctgtgcaacgtggacatcttcaaccccaagtacgactgcaagatcatgaccagcaagaccgacgtgagcagcagcgtgatcaccagcctgggcgccatcgtgagctgctacggcaagaccaagtgcaccgccagcaacaagaacaggggcatcatcaagaccttcagcaacggctgcgactacgtgagcaacaagggcgtggacaccgtgagcgtgggcaacaccctgtactacgtgaacaagcaggagggcaagagcctgtacgtgaagggcgagcccatcatcaacttctacgaccccctggtgttccccagcgacgagttcgacgccagcatcagccaggtgaacgagaagatcaaccagagcctggccttcatcaggaagagcgacgagctgctgcacaacgtgaacgccggcaagagcaccaccaacaccggcttcatcatcgtgatcatcctgatcgccgtgctgggcagcagcatgatcctggtgagcatcttcatcatcatcaagaagaccaagaagcagaccggcgccccccccgagctgagcggcgtgaccaacaacggcttcatcccccacagctgattaaaacagcggatgggtaccccaccatccgacccactgggtgtagtactctggtacttcgtacctttgtacgcctgttcttcccattgtacccttcctgaacttccaacccaagtaacgttagaagctcaacatttagtacaacaggaagcaccacatccagtggtgtttagtacaagcacttctgtttccccggagcgaggtataggctgtacccactgccaaaaacctttaaccgttatccgccaaccaactacgtaaaagctagtagtattatgtttttaactaggcgttcgatcaggtggatttcccctccactagtttggtcgatgaggctaggaattccccacgggtgaccgtgtcctagcctgcgtggcggccaacccagcttatgctgggacgcctttttatagacatggtgtgaagactcgcatgtgcttggttgtgattcctccggcccctgaatgcggctaaccttaaccctggagccttgtgtcacaaaccagtgatgataaggtcgtaatgagcaattccgggacgggaccgactactttgggtgtccgtgtttcttatttttcttattattgtcttatggtcacagcatatatataacatatactgtgatcatggagtcctaccttgttgatacctaccagggaattccttacacagctgctgtgcaagtggacctgattgaaaaggacctcctgcccgcctccctgaccatttggttccccctgttccaggccaacacacctcctgctgtcctgctggaccagctgaaaaccctcaccatcaccaccctgtatgcagcctctcagaatggccccatcctcaaggtgaatgccagcgcccagggggccgccatgagcgtgctccccaaaaagtttgaagtgaacgccaccgtggccttggatgaatattccaaactggagtttgacaagctcactgtgtgtgaggtgaagaccgtgtacctgaccacaatgaagccctatggcatggtgagcaaatttgtgagcagcgccaagtcagtgggcaagaaaacacatgatctcatcgccctgtgtgacttcatggacttggagaagaacacccctgtgaccattccagccttcatcaagtctgtgtccatcaaagaatctgaaagcgccacagtggaagctgccatctcctctgaggccgatcaggctctgacccaagccaaaattgccccctatgcaggcctgatcatgatcatgaccatgaacaaccccaagggcatcttcaagaagctgggggctgggacccaggtgattgtggagctgggcgcctacgtgcaggcagagagcatcagcaagatctgcaagacatggagccaccagggcacccgctacgtgctgaagagcaggtgattaaaacagcggatgggtaccccaccatccgacccactgggtgtagtactctggtacttcgtacctttgtacgcctgttcttcccattgtacccttcctgaacttccaacccaagtaacgttagaagctcaacatttagtacaacaggaagcaccacatccagtggtgtttagtacaagcacttctgtttccccggagcgaggtataggctgtacccactgccaaaaacctttaaccgttatccgccaaccaactacgtaaaagctagtagtattatgtttttaactaggcgttcgatcaggtggatttcccctccactagtttggtcgatgaggctaggaattccccacgggtgaccgtgtcctagcctgcgtggcggccaacccagcttatgctgggacgcctttttatagacatggtgtgaagactcgcatgtgcttggttgtgattcctccggcccctgaatgcggctaaccttaaccctggagccttgtgtcacaaaccagtgatgataaggtcgtaatgagcaattccgggacgggaccgactactttgggtgtccgtgtttcttatttttcttattattgtcttatggtcacagcatatatataacatatactgtgatcatggagagctacctggtggacacctaccagggcatcccctacaccgccgccgtgcaggtggacctgatcgagaaggacctgctgcccgccagcctgaccatctggttccccctgttccaggccaacaccccccccgccgtgctgctggaccagctgaagaccctgaccatcaccaccctgtacgccgccagccagaacggccccatcctgaaggtgaacgccagcgcccagggcgccgccatgagcgtgctgcccaagaagttcgaggtgaacgccaccgtggccctggacgagtacagcaagctggagttcgacaagctgaccgtgtgcgaggtgaagaccgtgtacctgaccaccatgaagccctacggcatggtgagcaagttcgtgagcagcgccaagagcgtgggcaagaagacccacgacctgatcgccctgtgcgacttcatggacctggagaagaacacccccgtgaccatccccgccttcatcaagagcgtgagcatcaaggagagcgagagcgccaccgtggaggccgccatcagcagcgaggccgaccaggccctgacccaggccaagatcgccccctacgccggcctgatcatgatcatgaccatgaacaaccccaagggcatcttcaagaagctgggcgccggcacccaggtgatcgtggagctgggcgcctacgtgcaggccgagagcatcagcaagatctgcaagacctggagccaccagggcaccaggtacgtgctgaagagcaggtaactcgagctggtactgcatgcacgcaatgctagctgcccctttcccgtcctgggtaccccgagtctcccccgacctcgggtcccaggtatgctcccacctccacctgccccactcaccacctctgctagttccagacacctcccaagcacgcagcaatgcagctcaaaacgcttagcctagccacacccccacgggaaacagcagtgattaacctttagcaataaacgaaagtttaactaagctatactaaccccagggttggtcaatttcgtgccagccacaccctggagctagcaaaaaaaaaaaaaaaaaaaaaaaaaaaaaagcatatgactaaaaaaaaaaaaaaaaaaaaaaaaaaaaaaaaaaaaaaaaaaaaaaaaaaaaaaaaaaaaaaaaaaaaaa

SEQ ID NO: 6 - DNA, 4772 bp, synthetic construct
  source 1..4772: mol_type = other DNA
aaataagagagaaaagaagagtaagaagaaatataagagccaccatggaactgctgatcctgaaggccaacgccatcaccaccatcctgaccgccgtgaccttctgttttgccagcggccagaacatcaccgaggaattctaccagagcacctgtagcgccgtgtccaagggctatctgagcgcccttagaaccggctggtacaccagcgtgatcaccatcgagctgagcaacatcaaagaaaacaagtgcaacggcaccgacgccaaagtgaagctgatcaagcaagagctggacaagtacaagaatgccgtgaccgaactgcagctgctgatgcagtctacccctgccaccaacaaccgggccagaagagaactgcccagattcatgaactacaccctgaacaacgccaaaaagaccaacgtgaccctgagcaagaagcggaagcggagattcctgggctttctgctcggagtgggaagcgccattgctagcggagtggccgtgtgtaaagtgctgcacctggaaggcgaagtgaacaagatcaagagcgccctgctgagcaccaacaaggccgtggtgtctctgtccaatggcgtgtccgtgctgaccttcaaggtgctggacctgaagaactacatcgacaaacagctgctgcccatcctgaacaagcagtcctgcagcatcagcaacatcgagacagtgatcgagttccagcagaagaacaaccggctgctggaaatcacccgcgagttctctgtgaatgccggcgtgaccacacctgtgtccacctacatgctgaccaacagcgagctgctgtccctgatcaacgacatgcccatcaccaacgaccagaaaaagctgatgagcaacaacgtgcagatcgtgcggcagcagagctacagcatcatgtgcattatcaaagaagaggtgctggcctacgtggtgcagctgcctctgtatggcgtgatcgataccccttgctggaagctgcacacaagccctctgtgcaccaccaacaccaaagagggctccaacatctgcctgaccagaaccgacagaggctggtactgcgataatgccggcagcgtctcattcttcccacaagccgagacatgcaaggtgcagagcaaccgggtgttctgcgacaccatgaacagcctgacactgccctccgaagtgaatctgtgcaacgtggacatcttcaaccctaagtacgactgcaagatcatgaccagcaagaccgacgtgtccagcagtgtgatcacctctctgggcgccatcgtgtcctgttacggcaagaccaagtgcaccgccagcaacaagaaccggggcatcatcaagaccttcagcaacggctgcgactacgtgtccaacaaaggcgtggacaccgtgtctgtgggcaacaccctgtactacgtgaacaaacaagagggcaagagcctgtacgtgaagggcgagcccatcatcaacttctacgaccctctggtgttccccagcgacgagttcgatgccagcatctcccaagtgaacgagaagatcaaccagagcctggccttcatcagaaagtccgatgagctgctgcacaacgtgaacgccggcaagtccaccaccaataccggcttcatcatcgtgatcatcctgattgccgtgctgggcagctccatgatcctggtgtccatctttatcatcatcaaaaagacgaagaagcagacaggcgcccctcctgaactgagcggcgtgacaaacaacggcttcattccccacagctgattaaaacagcggatgggtaccccaccatccgacccactgggtgtagtactctggtacttcgtacctttgtacgcctgttcttcccattgtacccttcctgaacttccaacccaagtaacgttagaagctcaacatttagtacaacaggaagcaccacatccagtggtgtttagtacaagcacttctgtttccccggagcgaggtataggctgtacccactgccaaaaacctttaaccgttatccgccaaccaactacgtaaaagctagtagtattatgtttttaactaggcgttcgatcaggtggatttcccctccactagtttggtcgatgaggctaggaattccccacgggtgaccgtgtcctagcctgcgtggcggccaacccagcttatgctgggacgcctttttatagacatggtgtgaagactcgcatgtgcttggttgtgattcctccggcccctgaatgcggctaaccttaaccctggagccttgtgtcacaaaccagtgatgataaggtcgtaatgagcaattccgggacgggaccgactactttgggtgtccgtgtttcttatttttcttattattgtcttatggtcacagcatatatataacatatactgtgatcatggagtcctaccttgttgatacctaccagggaattccttacacagctgctgtgcaagtggacctgattgaaaaggacctcctgcccgcctccctgaccatttggttccccctgttccaggccaacacacctcctgctgtcctgctggaccagctgaaaaccctcaccatcaccaccctgtatgcagcctctcagaatggccccatcctcaaggtgaatgccagcgcccagggggccgccatgagcgtgctccccaaaaagtttgaagtgaacgccaccgtggccttggatgaatattccaaactggagtttgacaagctcactgtgtgtgaggtgaagaccgtgtacctgaccacaatgaagccctatggcatggtgagcaaatttgtgagcagcgccaagtcagtgggcaagaaaacacatgatctcatcgccctgtgtgacttcatggacttggagaagaacacccctgtgaccattccagccttcatcaagtctgtgtccatcaaagaatctgaaagcgccacagtggaagctgccatctcctctgaggccgatcaggctctgacccaagccaaaattgccccctatgcaggcctgatcatgatcatgaccatgaacaaccccaagggcatcttcaagaagctgggggctgggacccaggtgattgtggagctgggcgcctacgtgcaggcagagagcatcagcaagatctgcaagacatggagccaccagggcacccgctacgtgctgaagagcaggtgattaaaacagcggatgggtaccccaccatccgacccactgggtgtagtactctggtacttcgtacctttgtacgcctgttcttcccattgtacccttcctgaacttccaacccaagtaacgttagaagctcaacatttagtacaacaggaagcaccacatccagtggtgtttagtacaagcacttctgtttccccggagcgaggtataggctgtacccactgccaaaaacctttaaccgttatccgccaaccaactacgtaaaagctagtagtattatgtttttaactaggcgttcgatcaggtggatttcccctccactagtttggtcgatgaggctaggaattccccacgggtgaccgtgtcctagcctgcgtggcggccaacccagcttatgctgggacgcctttttatagacatggtgtgaagactcgcatgtgcttggttgtgattcctccggcccctgaatgcggctaaccttaaccctggagccttgtgtcacaaaccagtgatgataaggtcgtaatgagcaattccgggacgggaccgactactttgggtgtccgtgtttcttatttttcttattattgtcttatggtcacagcatatatataacatatactgtgatcatggaaagctacctggtggatacctaccagggcatcccttacacagccgccgtgcaggttgacctgatcgagaaggatctgctgcctgccagcctgaccatctggttcccactgttccaggccaacacacctcctgccgttctgctggaccagctgaaaaccctgacaatcaccacactgtacgccgccagccagaatggccccatcctgaaagtgaatgccagcgctcaaggcgccgctatgagcgtgctgcccaagaaattcgaagtgaacgccacagtggccctggacgagtacagcaagctggaattcgacaagctgaccgtgtgcgaagtgaaaaccgtgtacctgaccaccatgaagccctacggcatggtgtccaagttcgtgtccagcgccaagagcgtgggcaagaaaacccacgatctgatcgccctgtgcgacttcatggacctggaaaagaacacccctgtgacaatccccgccttcatcaagtccgtgtctatcaaagagtccgagagcgccaccgtggaagccgccatttcttctgaagccgatcaggccctgacacaggccaagattgccccttatgccggcctgatcatgattatgaccatgaacaaccccaagggcatcttcaagaagctcggcgctggcacccaagtgatcgtggaactgggagcctatgtgcaggccgagagcatcagcaagatctgcaagacatggtcccaccagggcaccagatacgtgctgaagtccagatgagcggccgcttaattaagctgccttctgcggggcttgccttctggccatgcccttcttctctcccttgcacctgtacctcttggtctttgaataaagcctgagtaggaagaaaaaaaaaaaaaaaaaaaaaaaaaaaaagcatatgactaaaaaaaaaaaaaaaaaaaaaaaaaaaaaaaaaaaaaaaaaaaaaaaaaaaaaaaaaaaaaaaaaaaaaa